European Patent Application EP 4 566 613 A1, published June 11, 2025. Title: Therapeutic agent for Hunner-type interstitial cystitis containing DNA oligonucleotide selectively binding to IFN-γ. Applicant: TAGCYX Biotechnologies Inc. The sequence listing filed with the application follows.

SEQUENCE LISTING (4 sequences)

SEQ ID NO: 1 - DNA, 48 bp, synthetic construct
  source 1..48: mol_type = other DNA
  misc_feature 28: note = n is synthetic base; Ds(7-(2-thienyl)imidazo[4,5-b]pyridine)
  misc_feature 39: note = n is synthetic base; Ds(7-(2-thienyl)imidazo[4,5-b]pyridine)
cccgcccgggtccgcgaagcggtaggtntgggctaggcngctggcggg

SEQ ID NO: 2 - DNA, 57 bp, synthetic construct
  source 1..57: mol_type = other DNA
  misc_feature 28: note = n is synthetic base; Ds(7-(2-thienyl)imidazo[4,5-b]pyridine)
  misc_feature 39: note = n is synthetic base; Ds(7-(2-thienyl)imidazo[4,5-b]pyridine)
cccgcccgggtccgcgaagcggtaggtntgggctaggcngctggcgggcgcgaagcg

SEQ ID NO: 3 - DNA, 57 bp, synthetic construct
  source 1..57: mol_type = other DNA
  misc_feature 28: note = n is synthetic base; Ds(7-(2-thienyl)imidazo[4,5-b]pyridine)
  misc_feature 39: note = n is synthetic base; Ds(7-(2-thienyl)imidazo[4,5-b]pyridine)
  misc_feature 53: note = n is a natural base or an artificial base
cccgcccgggtccgcgaagcggtaggtntgggctaggcngctggcgggcgcgnagcg

SEQ ID NO: 4 - DNA, 62 bp, synthetic construct
  source 1..62: mol_type = other DNA
  misc_feature 14: note = n is synthetic base; Ds(7-(2-thienyl)imidazo[4,5-b]pyridine)
  misc_feature 26: note = n is synthetic base; Ds(7-(2-thienyl)imidazo[4,5-b]pyridine)
ggccggtacccganccacagtttatngttgtactagttttgcagggtctggcccgcgaagcg